European Patent Application EP 4 814 015 A1, published September 30, 2026. Title: 이량체 TCTP의 수용체인 CD300c 및 이의 용도. Applicant: 이화여자대학교 산학협력단. The sequence listing filed with the application follows.

SEQUENCE LISTING (66 sequences)

SEQ ID NO: 1 - protein, 172 aa, artificial sequence
MIIYRDLISHDEMFSDIYKIREIADGLCLEVEGKMVSRTEGNIDDSLIGGNASAEGPEGEGTESTVITGVDIVMNHHLQETSFTKEAYKKYIKDYMKSIKGKLEEQRPERVKPFMTGAAEQIKHILANFKNYQFFIGENMNPDGMVALLDYREDGVTPYMIFFKDGLEMEKC

SEQ ID NO: 2 - DNA, 489 bp, artificial sequence
  source 1..489: mol_type = other DNA
gatgagatgttctccgacatctacaagatccgggagatcgcggacgggttgtgcctggaggtggaggggaagatggtcagtaggacagaaggtaacattgatgactcgctcattggtggaaatgcctccgctgaaggccccgagggcgaaggtaccgaaagcacagtaatcactggtgtcgatattgtcatgaaccatcacctgcaggaaacaagtttcacaaaagaagcctacaagaagtacatcaaagattacatgaaatcaatcaaagggaaacttgaagaacagagaccagaaagagtaaaaccttttatgacaggggctgcagaacaaatcaagcacatccttgctaatttcaaaaactaccagttctttattggtgaaaacatgaatccagatggcatggttgctctattggactaccgtgaggatggtgtgaccccatatatgattttctttaaggatggtttagaaatggaaaaatgttaa

SEQ ID NO: 3 - protein, 224 aa, artificial sequence
MTARAWASWRSSALLLLLVPGYFPLSHPMTVAGPVGGSLSVQCRYEKEHRTLNKFWCRPPQILRCDKIVETKGSAGKRNGRVSIRDSPANLSFTVTLENLTEEDAGTYWCGVDTPWLRDFHDPIVEVEVSVFPAGTTTASSPQSSMGTSGPPTKLPVHTWPSVTRKDSPEPSPHPGSLFSNVRFLLLVLLELPLLLSMLGAVLWVNRPQRSSRSRQNWPKGENQ

SEQ ID NO: 4 - DNA, 672 bp, artificial sequence
  source 1..672: mol_type = other DNA
atgactgccagggcctgggcctcgtggcggtcttcagctctgctcctcctgcttgtcccaggctattttcctctgagccaccccatgaccgtggcgggccccgtggggggatccctgagtgtgcagtgtcgctatgagaaggaacacaggaccctcaacaaattctggtgcagaccaccacagattctccgatgtgacaagattgtggagaccaaagggtcagcagggaaaaggaatggccgagtgtccatcagggacagtcctgcaaacctcagcttcacagtgaccctggagaatctcacagaggaggacgcaggcacctactggtgtggggtggatacaccgtggctccgagactttcatgatcccattgtcgaggttgaggtgtccgtgttcccggccgggacgaccacagcctccagcccccagagctccatgggcacctcaggtcctcccacgaagctgcccgtgcacacctggcccagcgtgaccagaaaggacagccccgaacccagcccacaccctggctccctgttcagcaatgtccgcttcctgctcctggtcctcttggagctgcccctgctcctgagcatgctgggtgccgtcctctgggtgaacagacctcagagaagctctagaagcaggcagaattggcccaagggtgagaaccag

SEQ ID NO: 5 - DNA, 732 bp, artificial sequence
  source 1..732: mol_type = other DNA
gagctcgcactcacgcagtctccatcctccctgtctgcttctgtaggagacagagtcaccatcacttgccaagcgagtcacgacattagcaaatatttaaattggtatcaacagaaatcagggaaagcccctaagctcctgatctacgatgcgtccaatttggaaacaggagtcccgtcaaggttcagtggcagtggatctgggacagatttcactctcaccatcagcagtctgcaacctgaagattttgcaacttactactgtcaacagagttacagtaccccgctcactttcggcggagggaccaagctggagatcaaaggtggttcctctagatcttcctcctctggtggcggtggctcgggcggtggtgggcaggtgcagctgcaggagtcgggcccaggactggtgaagccttcacagaccctgtccctcacctgcactgtctctggtggctccatcagcagtggtagttactactggagctggatccggcagcccgccgggaagggactggagtggattgggcgtatttatagtagtgggagcaccaagtacaacccctccctcaagagccgagtcaccatatcaaaggacacgtccaagaatcagttctccctgaagctgagctctgtgaccgccgcggacacggccgtgtattactgtgcgagttcagtggctggacagaacgtcgactactggggccagggaaccctggtcaccgtctcctca

SEQ ID NO: 6 - protein, 244 aa, artificial sequence
ELALTQSPSSLSASVGDRVTITCQASHDISKYLNWYQQKSGKAPKLLIYDASNLETGVPSRFSGSGSGTDFTLTISSLQPEDFATYYCQQSYSTPLTFGGGTKLEIKGGSSRSSSSGGGGSGGGGQVQLQESGPGLVKPSQTLSLTCTVSGGSISSGSYYWSWIRQPAGKGLEWIGRIYSSGSTKYNPSLKSRVTISKDTSKNQFSLKLSSVTAADTAVYYCASSVAGQNVDYWGQGTLVTVSS

SEQ ID NO: 7 - protein, 103 aa, artificial sequence
TQSPSSLSASVGDRVTITCQASHDISKYLNWYQQKSGKAPKLLIYDASNLETGVPSRFSGSGSGTDFTLTISSLQPEDFATYYCQQSYSTPLTFGGGTKLEIK

SEQ ID NO: 8 - protein, 119 aa, artificial sequence
QVQLQESGPGLVKPSQTLSLTCTVSGGSISSGSYYWSWIRQPAGKGLEWIGRIYSSGSTKYNPSLKSRVTISKDTSKNQFSLKLSSVTAADTAVYYCASSVAGQNVDYWGQGTLVTVSS

SEQ ID NO: 9 - protein, 6 aa, artificial sequence
HDISKY

SEQ ID NO: 10 - skipped

SEQ ID NO: 11 - protein, 9 aa, artificial sequence
QQSYSTPLT

SEQ ID NO: 12 - protein, 10 aa, artificial sequence
GGSISSGSYY

SEQ ID NO: 13 - protein, 7 aa, artificial sequence
IYSSGST

SEQ ID NO: 14 - protein, 11 aa, artificial sequence
ASSVAGQNVDY

SEQ ID NO: 15 - protein, 18 aa, artificial sequence
GGSSRSSSSGGGGSGGGG

SEQ ID NO: 16 - DNA, 735 bp, artificial sequence
  source 1..735: mol_type = other DNA
gagctcgtgatgactcagtctccatcctccctgtctgcttctgtaggagacagagtcaccatcacttgccaagcgagtcacgacattagcaaatatttaaattggtatcaacagaaatcagggaaagcccctaagctcctgatctacgatgcgtccaatttggaaacaggagtcccgtcaaggttcagtggcagtggatctgcgacagatttcactctcaccatcagcagtctgcaacctgaagattttgcaacttactactgtcaacagagttacagtaccccgctcactttcggcggagggacacgactggagattaaaggtggttcctctagatcttcctcctctggtggcggtggctcgggcggtggtgggcagatcaccttgaaggagtctgggggaggcttggtacagcctggcaggtccctgagactctcctgtgcagccgctggattcacctttggtggttatgccatgcactgggtccggcaagctccagggaagggcctggagtgggtctcaggtattagttggaatggtggtgatatagcctatgcggactctgtgaagggccgattcaccatctccagagacaacgccaagaactccctgtatctgcaaatgaacagtctgggagctgaggacacggccttgtattactgtgcaaaatctagctggtggaagggagatgccttcgatatctggggccaagggacaatggtcaccgtctcctca

SEQ ID NO: 17 - protein, 245 aa, artificial sequence
ELVMTQSPSSLSASVGDRVTITCQASHDISKYLNWYQQKSGKAPKLLIYDASNLETGVPSRFSGSGSATDFTLTISSLQPEDFATYYCQQSYSTPLTFGGGTRLEIKGGSSRSSSSGGGGSGGGGQITLKESGGGLVQPGRSLRLSCAAAGFTFGGYAMHWVRQAPGKGLEWVSGISWNGGDIAYADSVKGRFTISRDNAKNSLYLQMNSLGAEDTALYYCAKSSWWKGDAFDIWGQGTMVTVSS

SEQ ID NO: 18 - protein, 104 aa, artificial sequence
MTQSPSSLSASVGDRVTITCQASHDISKYLNWYQQKSGKAPKLLIYDASNLETGVPSRFSGSGSATDFTLTISSLQPEDFATYYCQQSYSTPLTFGGGTRLEIK

SEQ ID NO: 19 - protein, 120 aa, artificial sequence
QITLKESGGGLVQPGRSLRLSCAAAGFTFGGYAMHWVRQAPGKGLEWVSGISWNGGDIAYADSVKGRFTISRDNAKNSLYLQMNSLGAEDTALYYCAKSSWWKGDAFDIWGQGTMVTVSS

SEQ ID NO: 20 - protein, 8 aa, artificial sequence
GFTFGGYA

SEQ ID NO: 21 - protein, 8 aa, artificial sequence
ISWNGGDI

SEQ ID NO: 22 - protein, 13 aa, artificial sequence
AKSSWWKGDAFDI

SEQ ID NO: 23 - DNA, 726 bp, artificial sequence
  source 1..726: mol_type = other DNA
gagctccagatgacccagtctccatcctccctgtctgcttctgtaggagacagagtcaccatcacttgccaagcaagtcacgacattagcaaatatttaaattggtatcaacagaaatcagggaaagcccctaagctcctgatctacgatgcgtccaatttggaaacaggagtcccgtcaaggttcagtggcagtggatctgggacagatttcactctcaccatcagcagtctgcaacctgaagattttgcaacttactactgtcaacagagttacagtaccccgctcactttcggcggagggaccaaggtgaccgtcctaggcggtggttcctctagatcttcctcctctggtggcggtggctcgggcggtggtgggcaggtgcagctgcaggagtcggggggaggcttggtacagcctggggggtccctgagactctcctgtgcagcctctggattcaactttaggaattatgccatgagctgggtccgccagactccagggaaggggctggagtgggtctcagctattaatggtagaggtgataccacatactacgcagactccgtgaagggccgattcaccatctccagagacaatgccaagaactcactgtatctgcaaatgaacagcctgagagccgaggacacggctgtatactactgtgcaagtggcgcctactattacaactactggggccagggaaccctggtcaccgtctcctca

SEQ ID NO: 24 - protein, 242 aa, artificial sequence
ELQMTQSPSSLSASVGDRVTITCQASHDISKYLNWYQQKSGKAPKLLIYDASNLETGVPSRFSGSGSGTDFTLTISSLQPEDFATYYCQQSYSTPLTFGGGTKVTVLGGGSSRSSSSGGGGSGGGGQVQLQESGGGLVQPGGSLRLSCAASGFNFRNYAMSWVRQTPGKGLEWVSAINGRGDTTYYADSVKGRFTISRDNAKNSLYLQMNSLRAEDTAVYYCASGAYYYNYWGQGTLVTVSS

SEQ ID NO: 25 - protein, 106 aa, artificial sequence
QMTQSPSSLSASVGDRVTITCQASHDISKYLNWYQQKSGKAPKLLIYDASNLETGVPSRFSGSGSGTDFTLTISSLQPEDFATYYCQQSYSTPLTFGGGTKVTVLG

SEQ ID NO: 26 - protein, 116 aa, artificial sequence
QVQLQESGGGLVQPGGSLRLSCAASGFNFRNYAMSWVRQTPGKGLEWVSAINGRGDTTYYADSVKGRFTISRDNAKNSLYLQMNSLRAEDTAVYYCASGAYYYNYWGQGTLVTVSS

SEQ ID NO: 27 - protein, 8 aa, artificial sequence
GFNFRNYA

SEQ ID NO: 28 - protein, 8 aa, artificial sequence
INGRGDTT

SEQ ID NO: 29 - protein, 9 aa, artificial sequence
ASGAYYYNY

SEQ ID NO: 30 - DNA, 738 bp, artificial sequence
  source 1..738: mol_type = other DNA
gagctcgtgctgactcagccaccctcaacgtctgcgacccccgggcagacggtcaccatctcctgttctggaagccactccaacatcgggactaatactgtgaactggtaccagcaactcccaggggcggcccccaagctcctcatctacagtgattcttttcgacccactggggtccctggccgattctctggctccaagtctggcacctcggcctccctggtcatcagtgggctccggtccgaggatgaggctgattattactgtgcagcatgggatgacagcctgaatggtccggtgttcggcggagggacccagctgaccgtcctcggcggtggttcctctagatcttcctcctctggtggcggtggctcgggcggtggtggggaggtgcagctggtgcagtctggagctgaggtgaagaagcctggggcctcagtaaaggtctcctgcaaggcttctggttacacctttaccagttatggtatcagctgggtgcgacaggcccctggacaagggcttgagtggatgggatggatcagtgtttacaatggtaacacaaactccgcacagaagctccagggcagagtcaccatgaccacagacacatccacgagcacagcctacatggagctgaggagcctgagatctgacgacacggccgtgtattactgtgcgagagaggatagcagctcgtttgactactggggccagggaaccctggtcaccgtctcctca

SEQ ID NO: 31 - protein, 246 aa, artificial sequence
ELVLTQPPSTSATPGQTVTISCSGSHSNIGTNTVNWYQQLPGAAPKLLIYSDSFRPTGVPGRFSGSKSGTSASLVISGLRSEDEADYYCAAWDDSLNGPVFGGGTQLTVLGGGSSRSSSSGGGGSGGGGEVQLVQSGAEVKKPGASVKVSCKASGYTFTSYGISWVRQAPGQGLEWMGWISVYNGNTNSAQKLQGRVTMTTDTSTSTAYMELRSLRSDDTAVYYCAREDSSSFDYWGQGTLVTVSS

SEQ ID NO: 32 - protein, 109 aa, artificial sequence
VLTQPPSTSATPGQTVTISCSGSHSNIGTNTVNWYQQLPGAAPKLLIYSDSFRPTGVPGRFSGSKSGTSASLVISGLRSEDEADYYCAAWDDSLNGPVFGGGTQLTVLG

SEQ ID NO: 33 - protein, 117 aa, artificial sequence
EVQLVQSGAEVKKPGASVKVSCKASGYTFTSYGISWVRQAPGQGLEWMGWISVYNGNTNSAQKLQGRVTMTTDTSTSTAYMELRSLRSDDTAVYYCAREDSSSFDYWGQGTLVTVSS

SEQ ID NO: 34 - protein, 8 aa, artificial sequence
HSNIGTNT

SEQ ID NO: 35 - skipped

SEQ ID NO: 36 - protein, 11 aa, artificial sequence
AAWDDSLNGPV

SEQ ID NO: 37 - protein, 8 aa, artificial sequence
GYTFTSYG

SEQ ID NO: 38 - protein, 8 aa, artificial sequence
ISVYNGNT

SEQ ID NO: 39 - protein, 10 aa, artificial sequence
AREDSSSFDY

SEQ ID NO: 40 - DNA, 729 bp, artificial sequence
  source 1..729: mol_type = other DNA
gagctcgtgatgactcagtctccatcctccctgtctgcttctgtaagagacagagtcaccatcacttgccaagcgagtcacgacattagcaaatatttaaattggtatcaacagaaatcagggaaagcccctaagctcctgatctacgatgcgtccaatttggaaacaggagtcccgtcaaggttcagtggcagtggatctgggacagatttcactctcaccatcagcagtctgcaacctgaagattttgcaacttactactgtcaacagagttacagtaccccgctcactttcggcggagggaccaaagtggatatcaaaggtggttcctctagatcttcctcctctggtggcggtggctcgggcggtggtgggcaggtgcagctgcaggagtcggggggaggcttggtacagcctggggggtccctgagactctcctgtgcagcctctggattcaactttaggaattatgccatgagctgggtccgccagactccagggaaggggctggagtgggtctcagctattaatggtagaggtgataccacatactacgcagactccgtgaaggaccgattcaccatctccagagacaattccaagaactcactgtatctacaaatgaacagcctgagagccgaggacacggccgtgtattactgtgcggccggtgcttatagcagctcgtttggcgaagagggccagggaaccctggtcatcgtctcctca

SEQ ID NO: 41 - protein, 243 aa, artificial sequence
ELVMTQSPSSLSASVRDRVTITCQASHDISKYLNWYQQKSGKAPKLLIYDASNLETGVPSRFSGSGSGTDFTLTISSLQPEDFATYYCQQSYSTPLTFGGGTKVDIKGGSSRSSSSGGGGSGGGGQVQLQESGGGLVQPGGSLRLSCAASGFNFRNYAMSWVRQTPGKGLEWVSAINGRGDTTYYADSVKDRFTISRDNSKNSLYLQMNSLRAEDTAVYYCAAGAYSSSFGEEGQGTLVIVSS

SEQ ID NO: 42 - protein, 104 aa, artificial sequence
MTQSPSSLSASVRDRVTITCQASHDISKYLNWYQQKSGKAPKLLIYDASNLETGVPSRFSGSGSGTDFTLTISSLQPEDFATYYCQQSYSTPLTFGGGTKVDIK

SEQ ID NO: 43 - protein, 118 aa, artificial sequence
QVQLQESGGGLVQPGGSLRLSCAASGFNFRNYAMSWVRQTPGKGLEWVSAINGRGDTTYYADSVKDRFTISRDNSKNSLYLQMNSLRAEDTAVYYCAAGAYSSSFGEEGQGTLVIVSS

SEQ ID NO: 44 - protein, 11 aa, artificial sequence
AAGAYSSSFGE

SEQ ID NO: 45 - DNA, 723 bp, artificial sequence
  source 1..723: mol_type = other DNA
gagctcacactcacgcagtctccatcctccctgtctgcttctgtaggagacagagtcaccatcacttgccaagcgagtcacgacattagcaaatatttaaattggtatcaacagaaatcagggaaagcccctaagctcctgatctacgatgcgtccaatttggaaacaggagtcccgtcaaggttcagtggcagtggatctgggacagatttcactctcaccatcagcagtctgcaacctgaagattttgcaatttactactgtcaacagagttacagtaccccgctcactttcggcggagggaccaagctggagatcaaaggtggttcctctagatcttcctcctctggtggcggtggctcgggcggtggtgggcaggtgcagctggtgcagtctgggggaggcgtggtccagcctgggaggtccctgagactctcctgtgcagcctctggattcaccttcagtagctatgccatgacctgggtccgccaggctccagggaaggggctggagtgggtctcagctattagtggtagtggtggtagcacatactacgcagactccgtgaagggccggttcaccatctccagagacaacgccaagaacacgctgtatctgcaaatgaacagtctgagagccgaggacacggctgtgtattactgtgcaagaggcccgtactactttgactactggggccagggaaccctggtcaccgtctcctca

SEQ ID NO: 46 - protein, 241 aa, artificial sequence
ELTLTQSPSSLSASVGDRVTITCQASHDISKYLNWYQQKSGKAPKLLIYDASNLETGVPSRFSGSGSGTDFTLTISSLQPEDFAIYYCQQSYSTPLTFGGGTKLEIKGGSSRSSSSGGGGSGGGGQVQLVQSGGGVVQPGRSLRLSCAASGFTFSSYAMTWVRQAPGKGLEWVSAISGSGGSTYYADSVKGRFTISRDNAKNTLYLQMNSLRAEDTAVYYCARGPYYFDYWGQGTLVTVSS

SEQ ID NO: 47 - protein, 103 aa, artificial sequence
TQSPSSLSASVGDRVTITCQASHDISKYLNWYQQKSGKAPKLLIYDASNLETGVPSRFSGSGSGTDFTLTISSLQPEDFAIYYCQQSYSTPLTFGGGTKLEIK

SEQ ID NO: 48 - protein, 116 aa, artificial sequence
QVQLVQSGGGVVQPGRSLRLSCAASGFTFSSYAMTWVRQAPGKGLEWVSAISGSGGSTYYADSVKGRFTISRDNAKNTLYLQMNSLRAEDTAVYYCARGPYYFDYWGQGTLVTVSS

SEQ ID NO: 49 - protein, 8 aa, artificial sequence
GFTFSSYA

SEQ ID NO: 50 - protein, 8 aa, artificial sequence
ISGSGGST

SEQ ID NO: 51 - protein, 9 aa, artificial sequence
ARGPYYFDY

SEQ ID NO: 52 - DNA, 723 bp, artificial sequence
  source 1..723: mol_type = other DNA
gagctccagatgacccagtctccatcctccctgtctgcttctgtaggagacagagtcaccatcacttgccaagcgagtcacgacattagcaaatatttaaattggtatcaacagaaatcagggaaagcccctaagctcctgatctacgatgcgtccaatttggaaacaggagtcccgtcaaggttcagtggcagtggatctgggacagatttcactctcaccatcagcagtctgcaacctgaagattttgcaacttactactgtcaacagagttacagtaccccgctcactttcggcggagggaccaaagtggatatcaaaggtggttcctctagatcttcctcctctggtggcggtggctcgggcggtggtgggcaggtgcagctacagcagtgggggggaggcctggtcaagcctggggggtccctgagactctcctgtgcagcctctggattcaactttaggaattatgccatgagctgggtccgccagactccagggaaggggctggagtgggtctcagctattaatggtagaggtgataccacatactacgcagactccgtgaagggccgattcaccatctccagagacaattccaaggacacactgtatctgcaaatgaacagtctgagagccgaggacacggctgtgtattactgtgcaagaggcccgtactactttgactacgggggccagggaaccctggtcaccgtctcctca

SEQ ID NO: 53 - protein, 241 aa, artificial sequence
ELQMTQSPSSLSASVGDRVTITCQASHDISKYLNWYQQKSGKAPKLLIYDASNLETGVPSRFSGSGSGTDFTLTISSLQPEDFATYYCQQSYSTPLTFGGGTKVDIKGGSSRSSSSGGGGSGGGGQVQLQQWGGGLVKPGGSLRLSCAASGFNFRNYAMSWVRQTPGKGLEWVSAINGRGDTTYYADSVKGRFTISRDNSKDTLYLQMNSLRAEDTAVYYCARGPYYFDYGGQGTLVTVSS

SEQ ID NO: 54 - protein, 105 aa, artificial sequence
QMTQSPSSLSASVGDRVTITCQASHDISKYLNWYQQKSGKAPKLLIYDASNLETGVPSRFSGSGSGTDFTLTISSLQPEDFATYYCQQSYSTPLTFGGGTKVDIK

SEQ ID NO: 55 - protein, 116 aa, artificial sequence
QVQLQQWGGGLVKPGGSLRLSCAASGFNFRNYAMSWVRQTPGKGLEWVSAINGRGDTTYYADSVKGRFTISRDNSKDTLYLQMNSLRAEDTAVYYCARGPYYFDYGGQGTLVTVSS

SEQ ID NO: 56 - protein, 229 aa, artificial sequence
MNPRVIRLWLPSAVLLSLVPGHFPVRGPSTVTGTVGESLSVSCQYEKKLKTKKKIWCKWKSNVLCKDIVKTSASEEARNGRVSIRDHPDNLTFTVTLENLTLEDAGTYMCMVDIGFFYDAYLQIDKSFKVEVFVVPGKPPFKGSRPGNGINILASPTSSAVHTQPNVTTDDTIPAPSPELRSLLSSPHFWILVSLKLPLFLSMLGALLWVNRPQRCSGGSSAWPCYENQ

SEQ ID NO: 57 - DNA, 729 bp, artificial sequence
  source 1..729: mol_type = other DNA
gagctcgccctgactcagcctccctccgtgtctgggtctcctggacagtcgatcaccctctcctgcactggaaccagcagtgatattggtgattataactatgtctcctggtaccaacaacacccaggcaaagcccccaaactcataatttatgaggtcaataatcggccctcaggggtttctattcgcttctctggctccaagtctggcaacacggcctccctgaccatctctgggctccaggctgaggatgaggctgattattactgcacttcatatacacccaggagcattgtcttcggcggagggacccagctgaccgtcctcggtggtggttcctctagatcttcctcctctggtggcggtggctcgggcggtggtggggaggtgcagctggtgcagtctgggggaggtgtggtacggcctggggggtccctgagactctcctgtgcagcctctggattcacctttgatgattatggcatgagctgggtccgccaagctccagggaaggggctggagtgggtctctggtattaattggaatggtggtagcacaatttatgcagactctgtgaagggccgattcatcatctccagagacaacgccaagaactccctgtatctgcaaatgaacagtctgagagccgaggacacggccctgtattattgtgttcgtggtcccgaccttgactactggggccagggaaccctgctcatcgtctcctca

SEQ ID NO: 58 - protein, 243 aa, artificial sequence
ELALTQPPSVSGSPGQSITLSCTGTSSDIGDYNYVSWYQQHPGKAPKLIIYEVNNRPSGVSIRFSGSKSGNTASLTISGLQAEDEADYYCTSYTPRSIVFGGGTQLTVLGGGSSRSSSSGGGGSGGGGEVQLVQSGGGVVRPGGSLRLSCAASGFTFDDYGMSWVRQAPGKGLEWVSGINWNGGSTIYADSVKGRFIISRDNAKNSLYLQMNSLRAEDTALYYCVRGPDLDYWGQGTLLIVSS

SEQ ID NO: 59 - protein, 110 aa, artificial sequence
ELALTQPPSVSGSPGQSITLSCTGTSSDIGDYNYVSWYQQHPGKAPKLIIYEVNNRPSGVSIRFSGSKSGNTASLTISGLQAEDEADYYCTSYTPRSIVFGGGTQLTVLG

SEQ ID NO: 60 - protein, 115 aa, artificial sequence
EVQLVQSGGGVVRPGGSLRLSCAASGFTFDDYGMSWVRQAPGKGLEWVSGINWNGGSTIYADSVKGRFIISRDNAKNSLYLQMNSLRAEDTALYYCVRGPDLDYWGQGTLLIVSS

SEQ ID NO: 61 - protein, 11 aa, artificial sequence
SSDIGDYNYVS

SEQ ID NO: 62 - protein, 4 aa, artificial sequence
EVNN

SEQ ID NO: 63 - protein, 7 aa, artificial sequence
TSYTPRS

SEQ ID NO: 64 - protein, 5 aa, artificial sequence
DYGMS

SEQ ID NO: 65 - protein, 9 aa, artificial sequence
GINWNGGST

SEQ ID NO: 66 - protein, 6 aa, artificial sequence
GPDLDY